European Patent Application EP 4 759 821 A1, published June 17, 2026. Title: Citrullinated SETDB1 polypeptide and use thereof in diagnosis of rheumatoid arthritis. Applicant: XIAMEN UNIVERSITY. Application CN PCT/CN2024/110642, filed August 8, 2024. The sequence listing filed with the application follows.

SEQUENCE LISTING (15 sequences)

SEQ ID NO: 1 - protein, 72 aa, synthetic construct
  source 1..72: note = SETDB1 MBD sequence
YRGKNPLLVPLLYDFRRMTARRRVNRKMGFHVIYKTPCGLCLRTMQEIERYLFETGCDFLFLEMFCLDPYVL

SEQ ID NO: 2 - protein, 23 aa, synthetic construct
  source 1..23: note = SETDB1 -Arg-4 amino acid sequence (aa5-27)
NPLLVPLLYDFRRMTARRRVNRK

SEQ ID NO: 3 - protein, 23 aa, synthetic construct
  source 1..23: note = SETDB1 -cit-4 amino acid sequence (aa5-27)
  MOD_RES 12..13: note = citrulline
  MOD_RES 17..19: note = citrulline
  MOD_RES 22: note = citrulline
NPLLVPLLYDFXXMTAXXXVNXK

SEQ ID NO: 4 - protein, 20 aa, synthetic construct
  source 1..20: note = SETDB1 -cit-4-truncated 1# amino acid sequence (aa8-27)
  MOD_RES 9..10: note = citrulline
  MOD_RES 14..16: note = citrulline
  MOD_RES 19: note = citrulline
LVPLLYDFXXMTAXXXVNXK

SEQ ID NO: 5 - protein, 16 aa, synthetic construct
  source 1..16: note = SETDB1 -cit-4-truncated 2# amino acid sequence (aa12-27)
  MOD_RES 5..6: note = citrulline
  MOD_RES 10..12: note = citrulline
  MOD_RES 15: note = citrulline
LYDFXXMTAXXXVNXK

SEQ ID NO: 6 - protein, 14 aa, synthetic construct
  source 1..14: note = SETDB1 -cit-4-truncated 3# amino acid sequence (aa14-27)
  MOD_RES 3..4: note = citrulline
  MOD_RES 8..10: note = citrulline
  MOD_RES 13: note = citrulline
DFXXMTAXXXVNXK

SEQ ID NO: 7 - protein, 12 aa, synthetic construct
  source 1..12: note = SETDB1 -cit-4-truncated 4# amino acid sequence (aa16-27)
  MOD_RES 1..2: note = citrulline
  MOD_RES 6..8: note = citrulline
  MOD_RES 11: note = citrulline
XXMTAXXXVNXK

SEQ ID NO: 8 - protein, 11 aa, synthetic construct
  source 1..11: note = SETDB1 -cit-4-truncated 5# amino acid sequence (aa16-26)
  MOD_RES 1..2: note = citrulline
  MOD_RES 6..8: note = citrulline
  MOD_RES 11: note = citrulline
XXMTAXXXVNX

SEQ ID NO: 9 - protein, 27 aa, synthetic construct
  source 1..27: note = SETDB1 -cit-4-lengthened 1# amino acid sequence (aa1-27)
  MOD_RES 2: note = citrulline
  MOD_RES 16..17: note = citrulline
  MOD_RES 21..23: note = citrulline
  MOD_RES 26: note = citrulline
YXGKNPLLVPLLYDFXXMTAXXXVNXK

SEQ ID NO: 10 - protein, 28 aa, synthetic construct
  source 1..28: note = SETDB1 -cit-4-lengthened 2# amino acid sequence (aa5-32)
  MOD_RES 12..13: note = citrulline
  MOD_RES 17..19: note = citrulline
  MOD_RES 22: note = citrulline
NPLLVPLLYDFXXMTAXXXVNXKMGFHV

SEQ ID NO: 11 - protein, 13 aa, synthetic construct
  source 1..13: note = cit-2 amino acid sequence
  MOD_RES 8: note = citrulline
EVKGPSGXSFCCE

SEQ ID NO: 12 - protein, 25 aa, synthetic construct
  source 1..25: note = cit-3 amino acid sequence
  MOD_RES 6: note = citrulline
  MOD_RES 11..12: note = citrulline
  MOD_RES 21: note = citrulline
  MOD_RES 23: note = citrulline
NMSVTXSNSLXXDSPPPPARXAXQE

SEQ ID NO: 13 - protein, 13 aa, synthetic construct
  source 1..13: note = cit-5 amino acid sequence
  MOD_RES 2: note = citrulline
  MOD_RES 8..10: note = citrulline
  MOD_RES 12: note = citrulline
PXMQIICXXXWXE

SEQ ID NO: 14 - protein, 10 aa, synthetic construct
  source 1..10: note = cit-8 amino acid sequence
  MOD_RES 4: note = citrulline
  MOD_RES 5: note = citrulline
ADMXXQMFAE

SEQ ID NO: 15 - protein, 11 aa, synthetic construct
  source 1..11: note = cit-9 amino acid sequence
  MOD_RES 7: note = citrulline
  MOD_RES 8: note = citrulline
  MOD_RES 10: note = citrulline
MGPGDFXXCXE